European Patent Application EP 4 194 552 A1, published June 14, 2023. Title: Nucleic acid structure. Applicant: CELLSPECT CO., LTD. THE SCHOOL CORPORATION KANSAI UNIVERSITY. The sequence listing filed with the application follows.

SEQUENCE LISTING (368 sequences)

SEQ ID NO: 1 - DNA, 38 bp, Artificial Sequence
  1s
cctaatttttttatcctgaatcttaccaacgctatttt

SEQ ID NO: 2 - DNA, 28 bp, Artificial Sequence
  2s
ttttacgagcgtctgcagcaccgttttt

SEQ ID NO: 3 - DNA, 32 bp, Artificial Sequence
  3s
caagtttgaatgaaaccatcgatattccagag

SEQ ID NO: 4 - DNA, 32 bp, Artificial Sequence
  4s
agctacaagccagttacaaaataaggccggaa

SEQ ID NO: 5 - DNA, 32 bp, Artificial Sequence
  5s
acgtcacccctttagcgtcagactacaacgcc

SEQ ID NO: 6 - DNA, 32 bp, Artificial Sequence
  6s
attatttaaagattagttgctattttgcaccc

SEQ ID NO: 7 - DNA, 32 bp, Artificial Sequence
  7s
ttttcatcccattaccattagcaaacagccat

SEQ ID NO: 8 - DNA, 22 bp, Artificial Sequence
  8s
ttgaagccttaaatctcccaat

SEQ ID NO: 9 - DNA, 28 bp, Artificial Sequence
  9s
ccaaataagaaacgatttagagccagca

SEQ ID NO: 10 - DNA, 28 bp, Artificial Sequence
  10
ttttaatcagtagcatagttagcgtttt

SEQ ID NO: 11 - DNA, 32 bp, Artificial Sequence
  11
tcgtcttttccacagacagccctcgacagaat

SEQ ID NO: 12 - DNA, 22 bp, Artificial Sequence
  12
tttttaacgatctaaagttttg

SEQ ID NO: 13 - DNA, 22 bp, Artificial Sequence
  13s
aaatcaccagtagcaggcattt

SEQ ID NO: 14 - DNA, 32 bp, Artificial Sequence
  14s
tgccatctgagccatttgggaatttttgttta

SEQ ID NO: 15 - DNA, 32 bp, Artificial Sequence
  15s
gcgttttaaatgaaaatagcagcctcaccgtc

SEQ ID NO: 16 - DNA, 32 bp, Artificial Sequence
  16s
accgactttttcataatcaaaatcctcatttt

SEQ ID NO: 17 - DNA, 42 bp, Artificial Sequence
  17s
taaaaacaatagaaggcttatccggtattctaagaacgcgag

SEQ ID NO: 18 - DNA, 28 bp, Artificial Sequence
  18s
aggtgaattatttacagagagaataaca

SEQ ID NO: 19 - DNA, 24 bp, Artificial Sequence
  19s
accggaacggaaattattcattaa

SEQ ID NO: 20 - DNA, 32 bp, Artificial Sequence
  20s
aatcagatgggaagcgcattagacgaaggtaa

SEQ ID NO: 21 - DNA, 32 bp, Artificial Sequence
  21s
atattgaccgcctccctcagagccagaaccgc

SEQ ID NO: 22 - DNA, 32 bp, Artificial Sequence
  22s
taactgaacattaccgcgcccaatagcaagca

SEQ ID NO: 23 - DNA, 32 bp, Artificial Sequence
  23
tgtatggggtcaccagtacaaactgtagcgcg

SEQ ID NO: 24 - DNA, 32 bp, Artificial Sequence
  24
tgtagcatccagacgttagtaaatgaattttc

SEQ ID NO: 25 - DNA, 32 bp, Artificial Sequence
  25s
cagaaccgaaccgattgagggagggggagaat

SEQ ID NO: 26 - DNA, 32 bp, Artificial Sequence
  26s
gtaggaatcaccctgaacaaagtccaaaaggg

SEQ ID NO: 27 - DNA, 32 bp, Artificial Sequence
  27s
cgacattcccaccctcagagccacccgtactc

SEQ ID NO: 28 - DNA, 32 bp, Artificial Sequence
  28s
attgagcgaagcaagccgtttttattttcatc

SEQ ID NO: 29 - DNA, 32 bp, Artificial Sequence
  29s
gagccgccttaccagcgccaaagaagagggta

SEQ ID NO: 30 - DNA, 32 bp, Artificial Sequence
  30s
tcgagaacctaatatcagagagatagaaaatt

SEQ ID NO: 31 - DNA, 32 bp, Artificial Sequence
  31s
catatggtaccagaaccaccaccatgatataa

SEQ ID NO: 32 - DNA, 32 bp, Artificial Sequence
  32s
agaattgagtattaaaccaagtaccgcactca

SEQ ID NO: 33 - DNA, 30 bp, Artificial Sequence
  33
tcggtcatgtaacactgagtttcattttgc

SEQ ID NO: 34 - DNA, 28 bp, Artificial Sequence
  34
cccatgtaccagcccccttattagcgtt

SEQ ID NO: 35 - DNA, 26 bp, Artificial Sequence
  35
taaacaactttcaacagtttcagcgg

SEQ ID NO: 36 - DNA, 32 bp, Artificial Sequence
  36s
gccagcatttttgtcacaatcaataacccaca

SEQ ID NO: 37 - DNA, 32 bp, Artificial Sequence
  37s
aagaacgggttaagcccaataataccacggaa

SEQ ID NO: 38 - DNA, 32 bp, Artificial Sequence
  38s
taagtttatgacaggaggttgaggagtaccag

SEQ ID NO: 39 - DNA, 32 bp, Artificial Sequence
  39s
aaacaatgtcggctgtctttccttatcattcc

SEQ ID NO: 40 - DNA, 32 bp, Artificial Sequence
  40s
acgattggaagaaacgcaaagacaagagcaag

SEQ ID NO: 41 - DNA, 24 bp, Artificial Sequence
  41
agtgagaagcaagcccaataggaa

SEQ ID NO: 42 - DNA, 32 bp, Artificial Sequence
  42s
atcaataaaaatagcaatagctataggtggca

SEQ ID NO: 43 - DNA, 32 bp, Artificial Sequence
  43s
acatataaccttgatattcacaaaagagaagg

SEQ ID NO: 44 - DNA, 32 bp, Artificial Sequence
  44s
agcccttttaatttacgagcatgtagaaacca

SEQ ID NO: 45 - DNA, 32 bp, Artificial Sequence
  45s
tcctcattgaaaatacatacataacttaccga

SEQ ID NO: 46 - DNA, 40 bp, Artificial Sequence
  46s
aaataatatcccatccttaagaaaagtaagcatatgttag

SEQ ID NO: 47 - DNA, 32 bp, Artificial Sequence
  47s
caaacgtaaaagccagaatggaaaacatgaaa

SEQ ID NO: 48 - DNA, 26 bp, Artificial Sequence
  48s
gaatcataataaggcgttaaataaga

SEQ ID NO: 49 - DNA, 32 bp, Artificial Sequence
  49s
aacaaagtaagtcctgaacaagaaaaacaccg

SEQ ID NO: 50 - DNA, 32 bp, Artificial Sequence
  50s
tctgaattactccttattacgcaggatagccg

SEQ ID NO: 51 - DNA, 32 bp, Artificial Sequence
  51s
tgtgataaattactagaaaaagcctttatcaa

SEQ ID NO: 52 - DNA, 28 bp, Artificial Sequence
  52
agccaccaccaccggaaccagagccacc

SEQ ID NO: 53 - DNA, 34 bp, Artificial Sequence
  53
cagggatatagaaaggaacaactaaaggaattgc

SEQ ID NO: 54 - DNA, 32 bp, Artificial Sequence
  54
gaataataattttttcgaaccgccaccctcag

SEQ ID NO: 55 - DNA, 32 bp, Artificial Sequence
  55s
caatagattaccagaaggaaaccgaactggca

SEQ ID NO: 56 - DNA, 32 bp, Artificial Sequence
  56s
tgattaagtaccgttccagtaagccccctgcc

SEQ ID NO: 57 - DNA, 32 bp, Artificial Sequence
  57
gctccaaatagtaccgccaccctcgccaccct

SEQ ID NO: 58 - DNA, 32 bp, Artificial Sequence
  58
caccctcaacgttgaaaatctccaaaaaaaag

SEQ ID NO: 59 - DNA, 32 bp, Artificial Sequence
  59s
atcatatgtttaatggtttgaaataccgaccg

SEQ ID NO: 60 - DNA, 32 bp, Artificial Sequence
  60s
caataataatgcagaacgcgcctgtgtttagt

SEQ ID NO: 61 - DNA, 32 bp, Artificial Sequence
  61
atcagcttcggaataggtgtatcacaccctca

SEQ ID NO: 62 - DNA, 32 bp, Artificial Sequence
  62
aggaggttaggagcctttaattgtatcggttt

SEQ ID NO: 63 - DNA, 32 bp, Artificial Sequence
  63s
tggcttttacggaatacccaaaagaggaaacg

SEQ ID NO: 64 - DNA, 32 bp, Artificial Sequence
  64s
gacctaaacgttatacaaattcttacaacatg

SEQ ID NO: 65 - DNA, 32 bp, Artificial Sequence
  65
agcttgatgtgccgtcgagagggtgagccgcc

SEQ ID NO: 66 - DNA, 32 bp, Artificial Sequence
  66
gtatagccgctttcgaggtgaatttcttaaac

SEQ ID NO: 67 - DNA, 32 bp, Artificial Sequence
  67s
ttcagctaaggtttaacgtcagataattgcgt

SEQ ID NO: 68 - DNA, 32 bp, Artificial Sequence
  68s
aaagccaaatattttagttaatttcatcttct

SEQ ID NO: 69 - DNA, 32 bp, Artificial Sequence
  69
aacaaccatagcggggttttgctccaggtcag

SEQ ID NO: 70 - DNA, 32 bp, Artificial Sequence
  70
gcggataaaccgatagttgcgccgacaatgac

SEQ ID NO: 71 - DNA, 32 bp, Artificial Sequence
  71s
agtaacagcagacgacgacaataaaccagtat

SEQ ID NO: 72 - DNA, 32 bp, Artificial Sequence
  72s
tttcaaatcgctcaacagtagggcgtaaagta

SEQ ID NO: 73 - DNA, 32 bp, Artificial Sequence
  73
cggtcgctaggctgagactcctcacaaataaa

SEQ ID NO: 74 - DNA, 32 bp, Artificial Sequence
  74
attaggattcgcccacgcataaccgatatatt

SEQ ID NO: 75 - DNA, 32 bp, Artificial Sequence
  75s
attctgtctaccttttacatcgggaaaattat

SEQ ID NO: 76 - DNA, 32 bp, Artificial Sequence
  76s
gaatcgccaagacaaagaacgcgagaaaactt

SEQ ID NO: 77 - DNA, 32 bp, Artificial Sequence
  77s
tatttcggaacctattattctgaagcgcagtc

SEQ ID NO: 78 - DNA, 24 bp, Artificial Sequence
  78s
gtattaaggaggcttgcagggagt

SEQ ID NO: 79 - DNA, 32 bp, Artificial Sequence
  79s
taacggataaagtaccgacaaaagttaattga

SEQ ID NO: 80 - DNA, 32 bp, Artificial Sequence
  80s
ccaatcgcatatttaacaacgccaagtaataa

SEQ ID NO: 81 - DNA, 32 bp, Artificial Sequence
  81c
ttgaatggtataaacagttaatgcgtcataca

SEQ ID NO: 82 - DNA, 40 bp, Artificial Sequence
  82s
taaaggccgcttttgcgaatacgtggcacagacaatattt

SEQ ID NO: 83 - DNA, 32 bp, Artificial Sequence
  83w
agattttcgatgatacaggagtgttgagtaac

SEQ ID NO: 84 - DNA, 32 bp, Artificial Sequence
  84w
taagttttaaaacagaaataaagagaatatac

SEQ ID NO: 85 - DNA, 32 bp, Artificial Sequence
  85c
gatagcccaacggggtcagtgcctactggtaa

SEQ ID NO: 86 - DNA, 32 bp, Artificial Sequence
  86c
agtgcccgctattagtctttaatgcgcgaact

SEQ ID NO: 87 - DNA, 32 bp, Artificial Sequence
  87w
ttgcacgtggtgaggcggtcagtacagaagat

SEQ ID NO: 88 - DNA, 32 bp, Artificial Sequence
  88w
gcctgcaatagaacctaccatatcagaaacaa

SEQ ID NO: 89 - DNA, 19 bp, Artificial Sequence
  89w
cgaaccaccagttaacacc

SEQ ID NO: 90 - DNA, 19 bp, Artificial Sequence
  90w
aaaacagataaaacatcgc

SEQ ID NO: 91 - DNA, 16 bp, Artificial Sequence
  91w
cattaaaaataccgaa

SEQ ID NO: 92 - DNA, 24 bp, Artificial Sequence
  92w
ggaagggtcagtgccacgctgaga

SEQ ID NO: 93 - DNA, 32 bp, Artificial Sequence
  93w
caaatgaagtttggattatacttcaataccaa

SEQ ID NO: 94 - DNA, 24 bp, Artificial Sequence
  94w
gcaaatcaacagttgagccagcag

SEQ ID NO: 95 - DNA, 16 bp, Artificial Sequence
  95w
aaggaattgaggaagg

SEQ ID NO: 96 - DNA, 32 bp, Artificial Sequence
  96w
tcctgattaaatctaaagcatcacaatatctg

SEQ ID NO: 97 - DNA, 32 bp, Artificial Sequence
  97w
acctcaaagatgatggcaattcatttattcat

SEQ ID NO: 98 - DNA, 32 bp, Artificial Sequence
  98w
ctaacaactatcaaaccctcaatccttgctga

SEQ ID NO: 99 - DNA, 32 bp, Artificial Sequence
  99w
gtcagttgttatctaaaatatctttaggagca

SEQ ID NO: 100 - DNA, 32 bp, Artificial Sequence
  100w
gattatcaacgttattaattttaataaatcct

SEQ ID NO: 101 - DNA, 32 bp, Artificial Sequence
  101w
gtaacattgagcggaattatcatctgatgaaa

SEQ ID NO: 102 - DNA, 32 bp, Artificial Sequence
  102w
taatacatattcgacaactcgtataagtttga

SEQ ID NO: 103 - DNA, 32 bp, Artificial Sequence
  103w
ttgcccgataatagattagagccgtcaataga

SEQ ID NO: 104 - DNA, 36 bp, Artificial Sequence
  104w
accagaagatcattttgcggaacattttttagactt

SEQ ID NO: 105 - DNA, 36 bp, Artificial Sequence
  105s
aacaatttaagaaaacaaaattaattttaagaaacc

SEQ ID NO: 106 - DNA, 28 bp, Artificial Sequence
  106w
tacaaacattgaggatttagaagttttt

SEQ ID NO: 107 - DNA, 32 bp, Artificial Sequence
  107s
caaacatccatttgaattacctttaacatagc

SEQ ID NO: 108 - DNA, 32 bp, Artificial Sequence
  108w
aaacagtacctgagcaaaagaagaatattcct

SEQ ID NO: 109 - DNA, 32 bp, Artificial Sequence
  109s
ttcaattacataaatcaatatatgctattaat

SEQ ID NO: 110 - DNA, 32 bp, Artificial Sequence
  110w
taaccttgatcgcgcagaggcgaacaatataa

SEQ ID NO: 111 - DNA, 32 bp, Artificial Sequence
  111s
gagaatattcgcctgattgctttgtgaataat

SEQ ID NO: 112 - DNA, 32 bp, Artificial Sequence
  112s
tttaggcactatatgtaaatgctgatgcaaat

SEQ ID NO: 113 - DNA, 32 bp, Artificial Sequence
  113s
gttacaaagaggcattttcgagccacatgtaa

SEQ ID NO: 114 - DNA, 32 bp, Artificial Sequence
  114s
ttatataacttctgtaaatcgtcgtgagtgaa

SEQ ID NO: 115 - DNA, 32 bp, Artificial Sequence
  115s
taattttcttttaacctccggcttaggttggg

SEQ ID NO: 116 - DNA, 32 bp, Artificial Sequence
  116s
gactacctccttagaatccttgaatttaatgg

SEQ ID NO: 117 - DNA, 32 bp, Artificial Sequence
  117s
gatagctttttatcaaaatcataggtctgaga

SEQ ID NO: 118 - DNA, 42 bp, Artificial Sequence
  118s
gagtcaatagtgaaagattaagacgctgagttttttacattt

SEQ ID NO: 119 - DNA, 42 bp, Artificial Sequence
  119s
accataaatcaaaagttcagaaaacgagaattttaaaatgtt

SEQ ID NO: 120 - DNA, 32 bp, Artificial Sequence
  120s
tttaaacaatcaggtctttaccctgactatta

SEQ ID NO: 121 - DNA, 32 bp, Artificial Sequence
  121s
tagtcagaattcattgaatccccccggaatcg

SEQ ID NO: 122 - DNA, 32 bp, Artificial Sequence
  122s
gagtagatagcaaagcggattgcatcaaaaag

SEQ ID NO: 123 - DNA, 28 bp, Artificial Sequence
  123w
agaccaggaaagaggacagatgaatttt

SEQ ID NO: 124 - DNA, 36 bp, Artificial Sequence
  124w
agtgaatatcaacgtaacaaagctttttcggtgtac

SEQ ID NO: 125 - DNA, 42 bp, Artificial Sequence
  125s
aaaagaagttttgcatagcgagaggcttttttttgctcattc

SEQ ID NO: 126 - DNA, 32 bp, Artificial Sequence
  126w
caactttgcgcataggctggctgaatattcat

SEQ ID NO: 127 - DNA, 32 bp, Artificial Sequence
  127w
tacccaaaaggcttgccctgacgagacgataa

SEQ ID NO: 128 - DNA, 24 bp, Artificial Sequence
  128s
aaaccaaacagagggggtaatagt

SEQ ID NO: 129 - DNA, 32 bp, Artificial Sequence
  129w
aagagtaacaatcataagggaaccgaactgac

SEQ ID NO: 130 - DNA, 32 bp, Artificial Sequence
  130w
agaacgagtcttgacaagaaccggccttcatc

SEQ ID NO: 131 - DNA, 32 bp, Artificial Sequence
  131w
tagactggccctcgtttaccagacgaaacacc

SEQ ID NO: 132 - DNA, 32 bp, Artificial Sequence
  132w
cagacggtacaaagtacaacggagttatacca

SEQ ID NO: 133 - DNA, 32 bp, Artificial Sequence
  133w
agcgcgaatagtaaattgggcttgagcaacac

SEQ ID NO: 134 - DNA, 32 bp, Artificial Sequence
  134s
tatcataaatagcgtccaatactgtcaaatgc

SEQ ID NO: 135 - DNA, 32 bp, Artificial Sequence
  135w
catcgcctatgttacttagccggaacgaggcg

SEQ ID NO: 136 - DNA, 32 bp, Artificial Sequence
  136w
taatttcactttgacccccagcgaatttgtat

SEQ ID NO: 137 - DNA, 32 bp, Artificial Sequence
  137w
tcataaattacgaggcatagtaagagatggtt

SEQ ID NO: 138 - DNA, 16 bp, Artificial Sequence
  138w
atccgcgacctgctcc

SEQ ID NO: 139 - DNA, 24 bp, Artificial Sequence
  139w
gataaattgtgtcgaaacactaaa

SEQ ID NO: 140 - DNA, 32 bp, Artificial Sequence
  140w
acactcatactttaatcattgtgataacgcca

SEQ ID NO: 141 - DNA, 32 bp, Artificial Sequence
  141s
aaaggaatttagtttgaccattagctgcgaac

SEQ ID NO: 142 - DNA, 24 bp, Artificial Sequence
  142w
atgcgattaaagaggcaaaagaat

SEQ ID NO: 143 - DNA, 32 bp, Artificial Sequence
  143s
cgcaaatgaactaatgcagatacaattacctt

SEQ ID NO: 144 - DNA, 16 bp, Artificial Sequence
  144w
agactttttcatgagg

SEQ ID NO: 145 - DNA, 19 bp, Artificial Sequence
  145w
aagtttccattgcaccaac

SEQ ID NO: 146 - DNA, 32 bp, Artificial Sequence
  146w
ctaaaacgttaagaactggctcattaggaata

SEQ ID NO: 147 - DNA, 32 bp, Artificial Sequence
  147s
ccacattcgtcaataacctgtttagtttcatt

SEQ ID NO: 148 - DNA, 19 bp, Artificial Sequence
  148w
aaaatacgttgaggactaa

SEQ ID NO: 149 - DNA, 32 bp, Artificial Sequence
  149w
tcaggacgtaatgccactacgaagaaacgggt

SEQ ID NO: 150 - DNA, 32 bp, Artificial Sequence
  150s
ttcatttgttcatcagttgagatttataccag

SEQ ID NO: 151 - DNA, 32 bp, Artificial Sequence
  151w
attaaagattgggaagaaaaatctattacagg

SEQ ID NO: 152 - DNA, 32 bp, Artificial Sequence
  152s
tagaaagagggcgcgagctgaaaattaaatat

SEQ ID NO: 153 - DNA, 32 bp, Artificial Sequence
  153w
aaaacgaatccagtttggaacaagcaaagggc

SEQ ID NO: 154 - DNA, 32 bp, Artificial Sequence
  154s
caattctactaacggaacaacattacgttaat

SEQ ID NO: 155 - DNA, 32 bp, Artificial Sequence
  155s
agtgttgttgaggggacgacgacacgtgcatc

SEQ ID NO: 156 - DNA, 32 bp, Artificial Sequence
  156s
tgccagttctaatagtagtagcatttgctgaa

SEQ ID NO: 157 - DNA, 32 bp, Artificial Sequence
  157c
cagaggctacgtggactccaacgtagtccact

SEQ ID NO: 158 - DNA, 32 bp, Artificial Sequence
  158c
gaaaaacctcggaacgagggtagcaacggcta

SEQ ID NO: 159 - DNA, 32 bp, Artificial Sequence
  159s
aataaatcatgggcgcatcgtaacgtatcggc

SEQ ID NO: 160 - DNA, 32 bp, Artificial Sequence
  160s
ctcaggaaaaagaatagcccgagagcccacta

SEQ ID NO: 161 - DNA, 32 bp, Artificial Sequence
  161c
agacagcagtctatcagggcgatgtagggttg

SEQ ID NO: 162 - DNA, 40 bp, Artificial Sequence
  162s
tgacctgaaagcgtaagggatcgtcaccctcagcagcgaa

SEQ ID NO: 163 - DNA, 40 bp, Artificial Sequence
  163s
gaattagcaaaattaatgaccgtaatgggatagctttccg

SEQ ID NO: 164 - DNA, 32 bp, Artificial Sequence
  164s
ataaatcagatcgcactccagccaggtcacgt

SEQ ID NO: 165 - DNA, 32 bp, Artificial Sequence
  165s
cgtgaaccatcacccaaatcaagtaatccctt

SEQ ID NO: 166 - DNA, 24 bp, Artificial Sequence
  166s
gtcgaggtagagatagaacccttc

SEQ ID NO: 167 - DNA, 32 bp, Artificial Sequence
  167s
gcaccgctgttccgaaatcggcaatttttggg

SEQ ID NO: 168 - DNA, 32 bp, Artificial Sequence
  168s
ctaaatcgcgtcggattctccgtgaggcaaag

SEQ ID NO: 169 - DNA, 32 bp, Artificial Sequence
  169
tggccaacgccgtaaagcactaaaatcctgtt

SEQ ID NO: 170 - DNA, 32 bp, Artificial Sequence
  170
ctaaagggcgaccagtaataaaagggacattc

SEQ ID NO: 171 - DNA, 32 bp, Artificial Sequence
  171s
cgccattcgccccagcaggcgaaatcggaacc

SEQ ID NO: 172 - DNA, 32 bp, Artificial Sequence
  172s
tgatggtgtctggtgccggaaaccggaacaaa

SEQ ID NO: 173 - DNA, 32 bp, Artificial Sequence
  173
cagtcacaagcccccgatttagagcggtccac

SEQ ID NO: 174 - DNA, 32 bp, Artificial Sequence
  174
ggaaagccgattatttacattggcagattcac

SEQ ID NO: 175 - DNA, 32 bp, Artificial Sequence
  175s
ggaagggcagagagttgcagcaagcttgacgg

SEQ ID NO: 176 - DNA, 32 bp, Artificial Sequence
  176s
gctggtttgccattcaggctgcgctgagcgag

SEQ ID NO: 177 - DNA, 32 bp, Artificial Sequence
  177
ctgaaatgggcgaacgtggcgagatcaccgcc

SEQ ID NO: 178 - DNA, 32 bp, Artificial Sequence
  178
gaagaaagacctacattttgacgctcaatcgt

SEQ ID NO: 179 - DNA, 32 bp, Artificial Sequence
  179s
tacgccagaacagctgattgccctaaggaagg

SEQ ID NO: 180 - DNA, 32 bp, Artificial Sequence
  180s
tggccctggatcggtgcgggcctcttcctgta

SEQ ID NO: 181 - DNA, 32 bp, Artificial Sequence
  181
atggaaatcgaaaggagcgggcgccaccagtg

SEQ ID NO: 182 - DNA, 32 bp, Artificial Sequence
  182
tggcaagtgccattgcaacaggaaaaacgctc

SEQ ID NO: 183 - DNA, 32 bp, Artificial Sequence
  183s
aggcgattgggtggtttttctttttagggcgc

SEQ ID NO: 184 - DNA, 32 bp, Artificial Sequence
  184s
agacgggcctggcgaaagggggatggaacgcc

SEQ ID NO: 185 - DNA, 32 bp, Artificial Sequence
  185
taccgccagtagcggtcacgctgctgcgtatt

SEQ ID NO: 186 - DNA, 32 bp, Artificial Sequence
  186
accacacctgctggtaatatccagaacaatat

SEQ ID NO: 187 - DNA, 32 bp, Artificial Sequence
  187s
ccagtcacgcggggagaggcggttgcgtaacc

SEQ ID NO: 188 - DNA, 32 bp, Artificial Sequence
  188s
gggcgccaaagttgggtaacgccattttgtta

SEQ ID NO: 189 - DNA, 32 bp, Artificial Sequence
  189
ctcaaactatcggcctcgccgcgcttaatgcg

SEQ ID NO: 190 - DNA, 34 bp, Artificial Sequence
  190
tatggttgtaacatcacttgcctgagtagaagaa

SEQ ID NO: 191 - DNA, 28 bp, Artificial Sequence
  191
ccgctacaggagctgcattaatgaatcg

SEQ ID NO: 192 - DNA, 32 bp, Artificial Sequence
  192s
atgcctgcggaaacctgtcgtgccgcgcgtac

SEQ ID NO: 193 - DNA, 24 bp, Artificial Sequence
  193s
gccaacgcgacgttgtaaaacgac

SEQ ID NO: 194 - DNA, 28 bp, Artificial Sequence
  194s
ggccagtgcctaaattgtaaacgttaat

SEQ ID NO: 195 - DNA, 42 bp, Artificial Sequence
  195s
attttgttttcaaaagggtgagaaaggccggagacagtcaaa

SEQ ID NO: 196 - DNA, 32 bp, Artificial Sequence
  196s
ggtaaagaaaaattcgcattaaatgggttttc

SEQ ID NO: 197 - DNA, 32 bp, Artificial Sequence
  197s
aatcagctaatgcaatgcctgagtaatgtgta

SEQ ID NO: 198 - DNA, 32 bp, Artificial Sequence
  198s
atattttacattttttaaccaatagtgctgca

SEQ ID NO: 199 - DNA, 32 bp, Artificial Sequence
  199s
atcaaaaagataaaaatttttagaaccctcat

SEQ ID NO: 200 - DNA, 32 bp, Artificial Sequence
  200s
aacgcaagtaattcgcgtctggccttcgctat

SEQ ID NO: 201 - DNA, 32 bp, Artificial Sequence
  201s
gccagcttttttgcgggagaagcctttatttc

SEQ ID NO: 202 - DNA, 32 bp, Artificial Sequence
  202s
tgtaatactcatcaacattaaatgaactgttg

SEQ ID NO: 203 - DNA, 32 bp, Artificial Sequence
  203s
taacaaccgttgtaccaaaaacattatgaccc

SEQ ID NO: 204 - DNA, 24 bp, Artificial Sequence
  204
attagtaactttgacgagcacgta

SEQ ID NO: 205 - DNA, 26 bp, Artificial Sequence
  205
ttaaccgttgtagcaatacttctttg

SEQ ID NO: 206 - DNA, 30 bp, Artificial Sequence
  206
aattgcgttcctcgttagaatcaacgcaaa

SEQ ID NO: 207 - DNA, 28 bp, Artificial Sequence
  207
taacgtgctttgcgctcactgcccgctt

SEQ ID NO: 208 - DNA, 32 bp, Artificial Sequence
  208s
tccagtcgaggtcgactctagaggccaaaaac

SEQ ID NO: 209 - DNA, 32 bp, Artificial Sequence
  209s
tcaccatctgtataagcaaatattaagcttgc

SEQ ID NO: 210 - DNA, 22 bp, Artificial Sequence
  210s
accgagctcgaattctcacatt

SEQ ID NO: 211 - DNA, 28 bp, Artificial Sequence
  211s
ttgataatcagaaaagccatccccgggt

SEQ ID NO: 212 - DNA, 34 bp, Artificial Sequence
  212s
aggaagataatatgatattcaaccgttctagctg

SEQ ID NO: 213 - DNA, 32 bp, Artificial Sequence
  213s
gagctaacgtaatcatggtcatagcatgtcaa

SEQ ID NO: 214 - DNA, 22 bp, Artificial Sequence
  214s
ataaattaatgccggaccccgg

SEQ ID NO: 215 - DNA, 32 bp, Artificial Sequence
  215s
tcatatgtagagggtagctatttttgagagat

SEQ ID NO: 216 - DNA, 32 bp, Artificial Sequence
  216s
tgtgtgaataaagcctggggtgccggaggccg

SEQ ID NO: 217 - DNA, 32 bp, Artificial Sequence
  217s
ctacaaaggtaatcgtaaaactagctgtttcc

SEQ ID NO: 218 - DNA, 32 bp, Artificial Sequence
  218s
ataaagtgattgttatccgctcacagagaatc

SEQ ID NO: 219 - DNA, 38 bp, Artificial Sequence
  219s
gatgaacggctatcaggtcattgcctgagagtcttttt

SEQ ID NO: 220 - DNA, 28 bp, Artificial Sequence
  220s
ttttggagcaaacaaattccacactttt

SEQ ID NO: 221 - DNA, 32 bp, Artificial Sequence
  221
tgtccatcgagcgggagctaaacataatgagt

SEQ ID NO: 222 - DNA, 32 bp, Artificial Sequence
  222
attaaagggtgaggccaccgagtaaaagagtc

SEQ ID NO: 223 - DNA, 32 bp, Artificial Sequence
  223s
cggcggatgcaataaagcctcagagcataaag

SEQ ID NO: 224 - DNA, 32 bp, Artificial Sequence
  224s
tggtgtagatacaggcaaggcaaagaggtcat

SEQ ID NO: 225 - DNA, 24 bp, Artificial Sequence
  225s
ttttgcggttaattgctccttttg

SEQ ID NO: 226 - DNA, 32 bp, Artificial Sequence
  226s
gagtacctatggcttagagcttaataacatcc

SEQ ID NO: 227 - DNA, 32 bp, Artificial Sequence
  227s
tataatgcaaactccaacaggtcaggattaga

SEQ ID NO: 228 - DNA, 32 bp, Artificial Sequence
  228s
ccggaagctgtagctcaacatgttggtggcat

SEQ ID NO: 229 - DNA, 32 bp, Artificial Sequence
  229s
gcaactaaattcgagcttcaaagcgaaccaga

SEQ ID NO: 230 - DNA, 32 bp, Artificial Sequence
  230s
gcgttttaagtacggtgtctggaagctatatt

SEQ ID NO: 231 - DNA, 32 bp, Artificial Sequence
  231s
ccatataagaagcccgaaagacttcaaatatc

SEQ ID NO: 232 - DNA, 32 bp, Artificial Sequence
  232s
attaagagcagttgattcccaattatacattt

SEQ ID NO: 233 - DNA, 32 bp, Artificial Sequence
  233
tataatcagattttagacaggaacccggaagc

SEQ ID NO: 234 - DNA, 22 bp, Artificial Sequence
  234
ttttaatcctgagaagtgtttt

SEQ ID NO: 235 - DNA, 28 bp, Artificial Sequence
  235
ttttaacatacgagggtacgccagtttt

SEQ ID NO: 236 - DNA, 34 bp, Artificial Sequence
  8s-2
acgtcaaagcgaacctcccgacttgcgggaggtt

SEQ ID NO: 237 - DNA, 40 bp, Artificial Sequence
  65long
tcttaaacagcttgatgtgccgtcgagagggtgagccgcc

SEQ ID NO: 238 - DNA, 40 bp, Artificial Sequence
  66shortTelo
gtatagccgctttcgaggtgaatttttttagggttagggt

SEQ ID NO: 239 - DNA, 40 bp, Artificial Sequence
  69long
acaatgacaacaaccatagcggggttttgctccaggtcag

SEQ ID NO: 240 - DNA, 40 bp, Artificial Sequence
  70shortTelo
gcggataaaccgatagttgcgccgtttttagggttagggt

SEQ ID NO: 241 - DNA, 40 bp, Artificial Sequence
  73long
gatatattcggtcgctaggctgagactcctcacaaataaa

SEQ ID NO: 242 - DNA, 40 bp, Artificial Sequence
  74shortTelo
attaggattcgcccacgcataacctttttagggttagggt

SEQ ID NO: 243 - DNA, 40 bp, Artificial Sequence
  78s-telo
gtattaaggaggcttgcagggagttttttagggttagggt

SEQ ID NO: 244 - DNA, 40 bp, Artificial Sequence
  166s-telo
gtcgaggtagagatagaacccttctttttagggttagggt

SEQ ID NO: 245 - DNA, 40 bp, Artificial Sequence
  169long
ggacattctggccaacgccgtaaagcactaaaatcctgtt

SEQ ID NO: 246 - DNA, 40 bp, Artificial Sequence
  170shortTelo
ctaaagggcgaccagtaataaaagtttttagggttagggt

SEQ ID NO: 247 - DNA, 40 bp, Artificial Sequence
  173long
agattcaccagtcacaagcccccgatttagagcggtccac

SEQ ID NO: 248 - DNA, 40 bp, Artificial Sequence
  174shortTelo
ggaaagccgattatttacattggctttttagggttagggt

SEQ ID NO: 249 - DNA, 40 bp, Artificial Sequence
  177long
tcaatcgtctgaaatgggcgaacgtggcgagatcaccgcc

SEQ ID NO: 250 - DNA, 40 bp, Artificial Sequence
  178shortTelo
gaagaaagacctacattttgacgctttttagggttagggt

SEQ ID NO: 251 - DNA, 40 bp, Artificial Sequence; identical to SEQ ID NO: 237
  65long

SEQ ID NO: 252 - DNA, 40 bp, Artificial Sequence; identical to SEQ ID NO: 238
  66shortTelo

SEQ ID NO: 253 - DNA, 40 bp, Artificial Sequence; identical to SEQ ID NO: 239
  69long

SEQ ID NO: 254 - DNA, 40 bp, Artificial Sequence; identical to SEQ ID NO: 240
  70shortTelo

SEQ ID NO: 255 - DNA, 54 bp, Artificial Sequence
  73LongCompM20
gtgcaggtagttttgatatattcggtcgctaggctgagactcctcacaaataaa

SEQ ID NO: 256 - DNA, 40 bp, Artificial Sequence; identical to SEQ ID NO: 242
  74shortTelo

SEQ ID NO: 257 - DNA, 40 bp, Artificial Sequence; identical to SEQ ID NO: 243
  78s-telo

SEQ ID NO: 258 - DNA, 40 bp, Artificial Sequence; identical to SEQ ID NO: 244
  166s-telo

SEQ ID NO: 259 - DNA, 56 bp, Artificial Sequence
  169LongCompM20
gtgcaggtagttttggaacatttctggccaacgccgtaaagcactaaaatcctgtt

SEQ ID NO: 260 - DNA, 40 bp, Artificial Sequence; identical to SEQ ID NO: 246
  170shortTelo

SEQ ID NO: 261 - DNA, 40 bp, Artificial Sequence; identical to SEQ ID NO: 247
  173long

SEQ ID NO: 262 - DNA, 40 bp, Artificial Sequence; identical to SEQ ID NO: 248
  174shortTelo

SEQ ID NO: 263 - DNA, 40 bp, Artificial Sequence; identical to SEQ ID NO: 249
  177long

SEQ ID NO: 264 - DNA, 40 bp, Artificial Sequence; identical to SEQ ID NO: 250
  178shortTelo

SEQ ID NO: 265 - DNA, 40 bp, Artificial Sequence
  81cLong
caatatttttgaatggtataaacagttaatgcgtcataca

SEQ ID NO: 266 - DNA, 73 bp, Artificial Sequence
  82sBothLongM20
gtgcaggtagtttttaaaggccgcttttgcgaatacgtggcacagattttctacctgcactataagcacttta

SEQ ID NO: 267 - DNA, 40 bp, Artificial Sequence
  85cLong
cgcgaactgatagcccaacggggtcagtgcctactggtaa

SEQ ID NO: 268 - DNA, 51 bp, Artificial Sequence
  86cShortMainM20
agtgcccgctattagtctttaatgttttctacctgcactataagcacttta

SEQ ID NO: 269 - DNA, 41 bp, Artificial Sequence
  157cLong
aaacggctacagaggctacgtggactccaacgtagtccact

SEQ ID NO: 270 - DNA, 51 bp, Artificial Sequence
  158cShortMainM20
gaaaaacctcggaacgagggtagcttttctacctgcactataagcacttta

SEQ ID NO: 271 - DNA, 40 bp, Artificial Sequence
  161cLong
gcagcgaaagacagcagtctatcagggcgatgtagggttg

SEQ ID NO: 272 - DNA, 73 bp, Artificial Sequence
  162sBothLongM20
gtgcaggtagtttttgacctgaaagcgtaagggatcgtcaccctcattttctacctgcactataagcacttta

SEQ ID NO: 273 - DNA, 7249 bp, Artificial Sequence
  M13mp18
aatgctactactattagtagaattgatgccaccttttcagctcgcgccccaaatgaaaatatagctaaacaggttattgaccatttgcgaaatgtatctaatggtcaaactaaatctactcgttcgcagaattgggaatcaactgttatatggaatgaaacttccagacaccgtactttagttgcatatttaaaacatgttgagctacagcattatattcagcaattaagctctaagccatccgcaaaaatgacctcttatcaaaaggagcaattaaaggtactctctaatcctgacctgttggagtttgcttccggtctggttcgctttgaagctcgaattaaaacgcgatatttgaagtctttcgggcttcctcttaatctttttgatgcaatccgctttgcttctgactataatagtcagggtaaagacctgatttttgatttatggtcattctcgttttctgaactgtttaaagcatttgagggggattcaatgaatatttatgacgattccgcagtattggacgctatccagtctaaacattttactattaccccctctggcaaaacttcttttgcaaaagcctctcgctattttggtttttatcgtcgtctggtaaacgagggttatgatagtgttgctcttactatgcctcgtaattccttttggcgttatgtatctgcattagttgaatgtggtattcctaaatctcaactgatgaatctttctacctgtaataatgttgttccgttagttcgttttattaacgtagatttttcttcccaacgtcctgactggtataatgagccagttcttaaaatcgcataaggtaattcacaatgattaaagttgaaattaaaccatctcaagcccaatttactactcgttctggtgtttctcgtcagggcaagccttattcactgaatgagcagctttgttacgttgatttgggtaatgaatatccggttcttgtcaagattactcttgatgaaggtcagccagcctatgcgcctggtctgtacaccgttcatctgtcctctttcaaagttggtcagttcggttcccttatgattgaccgtctgcgcctcgttccggctaagtaacatggagcaggtcgcggatttcgacacaatttatcaggcgatgatacaaatctccgttgtactttgtttcgcgcttggtataatcgctgggggtcaaagatgagtgttttagtgtattcttttgcctctttcgttttaggttggtgccttcgtagtggcattacgtattttacccgtttaatggaaacttcctcatgaaaaagtctttagtcctcaaagcctctgtagccgttgctaccctcgttccgatgctgtctttcgctgctgagggtgacgatcccgcaaaagcggcctttaactccctgcaagcctcagcgaccgaatatatcggttatgcgtgggcgatggttgttgtcattgtcggcgcaactatcggtatcaagctgtttaagaaattcacctcgaaagcaagctgataaaccgatacaattaaaggctccttttggagccttttttttggagattttcaacgtgaaaaaattattattcgcaattcctttagttgttcctttctattctcactccgctgaaactgttgaaagttgtttagcaaaatcccatacagaaaattcatttactaacgtctggaaagacgacaaaactttagatcgttacgctaactatgagggctgtctgtggaatgctacaggcgttgtagtttgtactggtgacgaaactcagtgttacggtacatgggttcctattgggcttgctatccctgaaaatgagggtggtggctctgagggtggcggttctgagggtggcggttctgagggtggcggtactaaacctcctgagtacggtgatacacctattccgggctatacttatatcaaccctctcgacggcacttatccgcctggtactgagcaaaaccccgctaatcctaatccttctcttgaggagtctcagcctcttaatactttcatgtttcagaataataggttccgaaataggcagggggcattaactgtttatacgggcactgttactcaaggcactgaccccgttaaaacttattaccagtacactcctgtatcatcaaaagccatgtatgacgcttactggaacggtaaattcagagactgcgctttccattctggctttaatgaggatttatttgtttgtgaatatcaaggccaatcgtctgacctgcctcaacctcctgtcaatgctggcggcggctctggtggtggttctggtggcggctctgagggtggtggctctgagggtggcggttctgagggtggcggctctgagggaggcggttccggtggtggctctggttccggtgattttgattatgaaaagatggcaaacgctaataagggggctatgaccgaaaatgccgatgaaaacgcgctacagtctgacgctaaaggcaaacttgattctgtcgctactgattacggtgctgctatcgatggtttcattggtgacgtttccggccttgctaatggtaatggtgctactggtgattttgctggctctaattcccaaatggctcaagtcggtgacggtgataattcacctttaatgaataatttccgtcaatatttaccttccctccctcaatcggttgaatgtcgcccttttgtctttggcgctggtaaaccatatgaattttctattgattgtgacaaaataaacttattccgtggtgtctttgcgtttcttttatatgttgccacctttatgtatgtattttctacgtttgctaacatactgcgtaataaggagtcttaatcatgccagttcttttgggtattccgttattattgcgtttcctcggtttccttctggtaactttgttcggctatctgcttacttttcttaaaaagggcttcggtaagatagctattgctatttcattgtttcttgctcttattattgggcttaactcaattcttgtgggttatctctctgatattagcgctcaattaccctctgactttgttcagggtgttcagttaattctcccgtctaatgcgcttccctgtttttatgttattctctctgtaaaggctgctattttcatttttgacgttaaacaaaaaatcgtttcttatttggattgggataaataatatggctgtttattttgtaactggcaaattaggctctggaaagacgctcgttagcgttggtaagattcaggataaaattgtagctgggtgcaaaatagcaactaatcttgatttaaggcttcaaaacctcccgcaagtcgggaggttcgctaaaacgcctcgcgttcttagaataccggataagccttctatatctgatttgcttgctattgggcgcggtaatgattcctacgatgaaaataaaaacggcttgcttgttctcgatgagtgcggtacttggtttaatacccgttcttggaatgataaggaaagacagccgattattgattggtttctacatgctcgtaaattaggatgggatattatttttcttgttcaggacttatctattgttgataaacaggcgcgttctgcattagctgaacatgttgtttattgtcgtcgtctggacagaattactttaccttttgtcggtactttatattctcttattactggctcgaaaatgcctctgcctaaattacatgttggcgttgttaaatatggcgattctcaattaagccctactgttgagcgttggctttatactggtaagaatttgtataacgcatatgatactaaacaggctttttctagtaattatgattccggtgtttattcttatttaacgccttatttatcacacggtcggtatttcaaaccattaaatttaggtcagaagatgaaattaactaaaatatatttgaaaaagttttctcgcgttctttgtcttgcgattggatttgcatcagcatttacatatagttatataacccaacctaagccggaggttaaaaaggtagtctctcagacctatgattttgataaattcactattgactcttctcagcgtcttaatctaagctatcgctatgttttcaaggattctaagggaaaattaattaatagcgacgatttacagaagcaaggttattcactcacatatattgatttatgtactgtttccattaaaaaaggtaattcaaatgaaattgttaaatgtaattaattttgttttcttgatgtttgtttcatcatcttcttttgctcaggtaattgaaatgaataattcgcctctgcgcgattttgtaacttggtattcaaagcaatcaggcgaatccgttattgtttctcccgatgtaaaaggtactgttactgtatattcatctgacgttaaacctgaaaatctacgcaatttctttatttctgttttacgtgcaaataattttgatatggtaggttctaacccttccattattcagaagtataatccaaacaatcaggattatattgatgaattgccatcatctgataatcaggaatatgatgataattccgctccttctggtggtttctttgttccgcaaaatgataatgttactcaaacttttaaaattaataacgttcgggcaaaggatttaatacgagttgtcgaattgtttgtaaagtctaatacttctaaatcctcaaatgtattatctattgacggctctaatctattagttgttagtgctcctaaagatattttagataaccttcctcaattcctttcaactgttgatttgccaactgaccagatattgattgagggtttgatatttgaggttcagcaaggtgatgctttagatttttcatttgctgctggctctcagcgtggcactgttgcaggcggtgttaatactgaccgcctcacctctgttttatcttctgctggtggttcgttcggtatttttaatggcgatgttttagggctatcagttcgcgcattaaagactaatagccattcaaaaatattgtctgtgccacgtattcttacgctttcaggtcagaagggttctatctctgttggccagaatgtcccttttattactggtcgtgtgactggtgaatctgccaatgtaaataatccatttcagacgattgagcgtcaaaatgtaggtatttccatgagcgtttttcctgttgcaatggctggcggtaatattgttctggatattaccagcaaggccgatagtttgagttcttctactcaggcaagtgatgttattactaatcaaagaagtattgctacaacggttaatttgcgtgatggacagactcttttactcggtggcctcactgattataaaaacacttctcaggattctggcgtaccgttcctgtctaaaatccctttaatcggcctcctgtttagctcccgctctgattctaacgaggaaagcacgttatacgtgctcgtcaaagcaaccatagtacgcgccctgtagcggcgcattaagcgcggcgggtgtggtggttacgcgcagcgtgaccgctacacttgccagcgccctagcgcccgctcctttcgctttcttcccttcctttctcgccacgttcgccggctttccccgtcaagctctaaatcgggggctccctttagggttccgatttagtgctttacggcacctcgaccccaaaaaacttgatttgggtgatggttcacgtagtgggccatcgccctgatagacggtttttcgccctttgacgttggagtccacgttctttaatagtggactcttgttccaaactggaacaacactcaaccctatctcgggctattcttttgatttataagggattttgccgatttcggaaccaccatcaaacaggattttcgcctgctggggcaaaccagcgtggaccgcttgctgcaactctctcagggccaggcggtgaagggcaatcagctgttgcccgtctcactggtgaaaagaaaaaccaccctggcgcccaatacgcaaaccgcctctccccgcgcgttggccgattcattaatgcagctggcacgacaggtttcccgactggaaagcgggcagtgagcgcaacgcaattaatgtgagttagctcactcattaggcaccccaggctttacactttatgcttccggctcgtatgttgtgtggaattgtgagcggataacaatttcacacaggaaacagctatgaccatgattacgaattcgagctcggtacccggggatcctctagagtcgacctgcaggcatgcaagcttggcactggccgtcgttttacaacgtcgtgactgggaaaaccctggcgttacccaacttaatcgccttgcagcacatccccctttcgccagctggcgtaatagcgaagaggcccgcaccgatcgcccttcccaacagttgcgcagcctgaatggcgaatggcgctttgcctggtttccggcaccagaagcggtgccggaaagctggctggagtgcgatcttcctgaggccgatactgtcgtcgtcccctcaaactggcagatgcacggttacgatgcgcccatctacaccaacgtgacctatcccattacggtcaatccgccgtttgttcccacggagaatccgacgggttgttactcgctcacatttaatgttgatgaaagctggctacaggaaggccagacgcgaattatttttgatggcgttcctattggttaaaaaatgagctgatttaacaaaaatttaatgcgaattttaacaaaatattaacgtttacaatttaaatatttgcttatacaatcttcctgtttttggggcttttctgattatcaaccggggtacatatgattgacatgctagttttacgattaccgttcatcgattctcttgtttgctccagactctcaggcaatgacctgatagcctttgtagatctctcaaaaatagctaccctctccggcattaatttatcagctagaacggttgaatatcatattgatggtgatttgactgtctccggcctttctcacccttttgaatctttacctacacattactcaggcattgcatttaaaatatatgagggttctaaaaatttttatccttgcgttgaaataaaggcttctcccgcaaaagtattacagggtcataatgtttttggtacaaccgatttagctttatgctctgaggctttattgcttaattttgctaattctttgccttgcctgtatgatttattggatgtt

SEQ ID NO: 274 - RNA, 23 nt, Homo sapiens
uaaagugcuuauagugcagguag

SEQ ID NO: 275 - DNA, 40 bp, Artificial Sequence; identical to SEQ ID NO: 237
  65long

SEQ ID NO: 276 - DNA, 40 bp, Artificial Sequence; identical to SEQ ID NO: 238
  66shortTelo

SEQ ID NO: 277 - DNA, 40 bp, Artificial Sequence; identical to SEQ ID NO: 239
  69long

SEQ ID NO: 278 - DNA, 40 bp, Artificial Sequence; identical to SEQ ID NO: 240
  70shortTelo

SEQ ID NO: 279 - DNA, 53 bp, Artificial Sequence
  73LongCompCF509
cagttcgagttttgatatattcggtcgctaggctgagactcctcacaaataaa

SEQ ID NO: 280 - DNA, 40 bp, Artificial Sequence; identical to SEQ ID NO: 242
  74shortTelo

SEQ ID NO: 281 - DNA, 40 bp, Artificial Sequence; identical to SEQ ID NO: 243
  78s-telo

SEQ ID NO: 282 - DNA, 40 bp, Artificial Sequence; identical to SEQ ID NO: 244
  166s-telo

SEQ ID NO: 283 - DNA, 55 bp, Artificial Sequence
  169LongCompCF509
cagttcgagttttggaacatttctggccaacgccgtaaagcactaaaatcctgtt

SEQ ID NO: 284 - DNA, 40 bp, Artificial Sequence; identical to SEQ ID NO: 246
  170shortTelo

SEQ ID NO: 285 - DNA, 40 bp, Artificial Sequence; identical to SEQ ID NO: 247
  173long

SEQ ID NO: 286 - DNA, 40 bp, Artificial Sequence; identical to SEQ ID NO: 248
  174shortTelo

SEQ ID NO: 287 - DNA, 40 bp, Artificial Sequence; identical to SEQ ID NO: 249
  177long

SEQ ID NO: 288 - DNA, 40 bp, Artificial Sequence; identical to SEQ ID NO: 250
  178shortTelo

SEQ ID NO: 289 - DNA, 40 bp, Artificial Sequence; identical to SEQ ID NO: 265
  81cLong

SEQ ID NO: 290 - DNA, 68 bp, Artificial Sequence
  82sBothLongCF509
cagttcgagtttttaaaggccgcttttgcgaatacgtggcacagattttctcgaactgcacctcatgg

SEQ ID NO: 291 - DNA, 40 bp, Artificial Sequence; identical to SEQ ID NO: 267
  85cLong

SEQ ID NO: 292 - DNA, 47 bp, Artificial Sequence
  86cShortCF509
agtgcccgctattagtctttaatgttttctcgaactgcacctcatgg

SEQ ID NO: 293 - DNA, 41 bp, Artificial Sequence; identical to SEQ ID NO: 269
  157cLong

SEQ ID NO: 294 - DNA, 47 bp, Artificial Sequence
  158cShortCF509
gaaaaacctcggaacgagggtagcttttctcgaactgcacctcatgg

SEQ ID NO: 295 - DNA, 40 bp, Artificial Sequence; identical to SEQ ID NO: 271
  161cLong

SEQ ID NO: 296 - DNA, 68 bp, Artificial Sequence
  162sBothLongCF509
cagttcgagtttttgacctgaaagcgtaagggatcgtcaccctcattttctcgaactgcacctcatgg

SEQ ID NO: 297 - DNA, 19 bp, Artificial Sequence
  R509
ccatgaggtgcagttcgag

SEQ ID NO: 298 - DNA, 40 bp, Artificial Sequence; identical to SEQ ID NO: 237
  65long

SEQ ID NO: 299 - DNA, 40 bp, Artificial Sequence; identical to SEQ ID NO: 238
  66shortTelo

SEQ ID NO: 300 - DNA, 40 bp, Artificial Sequence; identical to SEQ ID NO: 239
  69long

SEQ ID NO: 301 - DNA, 40 bp, Artificial Sequence; identical to SEQ ID NO: 240
  70shortTelo

SEQ ID NO: 302 - DNA, 54 bp, Artificial Sequence
  73LongCompN1
aacattgccattttgatatattcggtcgctaggctgagactcctcacaaataaa

SEQ ID NO: 303 - DNA, 40 bp, Artificial Sequence; identical to SEQ ID NO: 242
  74shortTelo

SEQ ID NO: 304 - DNA, 40 bp, Artificial Sequence; identical to SEQ ID NO: 243
  78s-telo

SEQ ID NO: 305 - DNA, 40 bp, Artificial Sequence; identical to SEQ ID NO: 244
  166s-telo

SEQ ID NO: 306 - DNA, 54 bp, Artificial Sequence
  169LongCompN1
aacattgccattttggacattctggccaacgccgtaaagcactaaaatcctgtt

SEQ ID NO: 307 - DNA, 40 bp, Artificial Sequence; identical to SEQ ID NO: 246
  170shortTelo

SEQ ID NO: 308 - DNA, 40 bp, Artificial Sequence; identical to SEQ ID NO: 247
  173long

SEQ ID NO: 309 - DNA, 40 bp, Artificial Sequence; identical to SEQ ID NO: 248
  174shortTelo

SEQ ID NO: 310 - DNA, 40 bp, Artificial Sequence; identical to SEQ ID NO: 249
  177long

SEQ ID NO: 311 - DNA, 40 bp, Artificial Sequence; identical to SEQ ID NO: 250
  178shortTelo

SEQ ID NO: 312 - DNA, 40 bp, Artificial Sequence; identical to SEQ ID NO: 265
  81cLong

SEQ ID NO: 313 - DNA, 75 bp, Artificial Sequence
  82sBothLongN1
aacattgccatttttaaaggccgcttttgcgaatacgtggcacagatttttggcaatgttgttccttgaggaagt

SEQ ID NO: 314 - DNA, 40 bp, Artificial Sequence; identical to SEQ ID NO: 267
  85cLong

SEQ ID NO: 315 - DNA, 53 bp, Artificial Sequence
  86cShortN1
agtgcccgctattagtctttaatgtttttggcaatgttgttccttgaggaagt

SEQ ID NO: 316 - DNA, 41 bp, Artificial Sequence; identical to SEQ ID NO: 269
  157cLong

SEQ ID NO: 317 - DNA, 53 bp, Artificial Sequence
  158cShortN1
gaaaaacctcggaacgagggtagctttttggcaatgttgttccttgaggaagt

SEQ ID NO: 318 - DNA, 40 bp, Artificial Sequence; identical to SEQ ID NO: 271
  161cLong

SEQ ID NO: 319 - DNA, 75 bp, Artificial Sequence
  162sBothLongN1
aacattgccatttttgacctgaaagcgtaagggatcgtcaccctcatttttggcaatgttgttccttgaggaagt

SEQ ID NO: 320 - DNA, 25 bp, Artificial Sequence
  N1
acttcctcaaggaacaacattgcca

SEQ ID NO: 321 - DNA, 40 bp, Artificial Sequence; identical to SEQ ID NO: 237
  65long

SEQ ID NO: 322 - DNA, 40 bp, Artificial Sequence; identical to SEQ ID NO: 238
  66shortTelo

SEQ ID NO: 323 - DNA, 40 bp, Artificial Sequence; identical to SEQ ID NO: 239
  69long

SEQ ID NO: 324 - DNA, 40 bp, Artificial Sequence; identical to SEQ ID NO: 240
  70shortTelo

SEQ ID NO: 325 - DNA, 54 bp, Artificial Sequence
  73LongCompHD1T1
acaccaacctttttgatatattcggtcgctaggctgagactcctcacaaataaa

SEQ ID NO: 326 - DNA, 40 bp, Artificial Sequence; identical to SEQ ID NO: 242
  74shortTelo

SEQ ID NO: 327 - DNA, 40 bp, Artificial Sequence; identical to SEQ ID NO: 243
  78s-telo

SEQ ID NO: 328 - DNA, 40 bp, Artificial Sequence; identical to SEQ ID NO: 244
  166s-telo

SEQ ID NO: 329 - DNA, 54 bp, Artificial Sequence
  169LongCompHD1T1
acaccaacctttttggacattctggccaacgccgtaaagcactaaaatcctgtt

SEQ ID NO: 330 - DNA, 40 bp, Artificial Sequence; identical to SEQ ID NO: 246
  170shortTelo

SEQ ID NO: 331 - DNA, 40 bp, Artificial Sequence; identical to SEQ ID NO: 247
  173long

SEQ ID NO: 332 - DNA, 40 bp, Artificial Sequence; identical to SEQ ID NO: 248
  174shortTelo

SEQ ID NO: 333 - DNA, 40 bp, Artificial Sequence; identical to SEQ ID NO: 249
  177long

SEQ ID NO: 334 - DNA, 40 bp, Artificial Sequence; identical to SEQ ID NO: 250
  178shortTelo

SEQ ID NO: 335 - DNA, 40 bp, Artificial Sequence; identical to SEQ ID NO: 265
  81cLong

SEQ ID NO: 336 - DNA, 71 bp, Artificial Sequence
  82sBothLongHD1T1
acaccaaccttttttaaaggccgcttttgcgaatacgtggcacagatttgtggttggtgtggttggtcata

SEQ ID NO: 337 - DNA, 40 bp, Artificial Sequence; identical to SEQ ID NO: 267
  85cLong

SEQ ID NO: 338 - DNA, 57 bp, Artificial Sequence
  86cShortHD1T1
agtgcccgctattagtctttaatgttttagtccgtggtagggcaggttggggtgact

SEQ ID NO: 339 - DNA, 41 bp, Artificial Sequence; identical to SEQ ID NO: 269
  157cLong

SEQ ID NO: 340 - DNA, 57 bp, Artificial Sequence
  158cShortHD1T1
gaaaaacctcggaacgagggtagcttttagtccgtggtagggcaggttggggtgact

SEQ ID NO: 341 - DNA, 40 bp, Artificial Sequence; identical to SEQ ID NO: 271
  161cLong

SEQ ID NO: 342 - DNA, 71 bp, Artificial Sequence
  162sBothLongHD1T1
acaccaaccttttttgacctgaaagcgtaagggatcgtcaccctcatttgtggttggtgtggttggtcata

SEQ ID NO: 343 - DNA, 25 bp, Artificial Sequence
  HD1
tttgtggttggtgtggttggtcata

SEQ ID NO: 344 - DNA, 20 bp, Artificial Sequence
  R29142
gttcctggtccccaaaattt

SEQ ID NO: 345 - DNA, 40 bp, Artificial Sequence; identical to SEQ ID NO: 237
  65long

SEQ ID NO: 346 - DNA, 40 bp, Artificial Sequence; identical to SEQ ID NO: 238
  66shortTelo

SEQ ID NO: 347 - DNA, 40 bp, Artificial Sequence; identical to SEQ ID NO: 239
  69long

SEQ ID NO: 348 - DNA, 40 bp, Artificial Sequence; identical to SEQ ID NO: 240
  70shortTelo

SEQ ID NO: 349 - DNA, 54 bp, Artificial Sequence; identical to SEQ ID NO: 255
  73LongCompM20

SEQ ID NO: 350 - DNA, 40 bp, Artificial Sequence; identical to SEQ ID NO: 242
  74shortTelo

SEQ ID NO: 351 - DNA, 40 bp, Artificial Sequence; identical to SEQ ID NO: 243
  78s-telo

SEQ ID NO: 352 - DNA, 40 bp, Artificial Sequence; identical to SEQ ID NO: 244
  166s-telo

SEQ ID NO: 353 - DNA, 56 bp, Artificial Sequence; identical to SEQ ID NO: 259
  169LongCompM20

SEQ ID NO: 354 - DNA, 40 bp, Artificial Sequence; identical to SEQ ID NO: 246
  170shortTelo

SEQ ID NO: 355 - DNA, 40 bp, Artificial Sequence; identical to SEQ ID NO: 247
  173long

SEQ ID NO: 356 - DNA, 40 bp, Artificial Sequence; identical to SEQ ID NO: 248
  174shortTelo

SEQ ID NO: 357 - DNA, 40 bp, Artificial Sequence; identical to SEQ ID NO: 249
  177long

SEQ ID NO: 358 - DNA, 40 bp, Artificial Sequence; identical to SEQ ID NO: 250
  178shortTelo

SEQ ID NO: 359 - DNA, 40 bp, Artificial Sequence; identical to SEQ ID NO: 265
  81cLong

SEQ ID NO: 360 - DNA, 73 bp, Artificial Sequence; identical to SEQ ID NO: 266
  82sBothLongM20

SEQ ID NO: 361 - DNA, 40 bp, Artificial Sequence; identical to SEQ ID NO: 267
  85cLong

SEQ ID NO: 362 - DNA, 51 bp, Artificial Sequence; identical to SEQ ID NO: 268
  86cShortMainM20

SEQ ID NO: 363 - DNA, 41 bp, Artificial Sequence; identical to SEQ ID NO: 269
  157cLong

SEQ ID NO: 364 - DNA, 51 bp, Artificial Sequence; identical to SEQ ID NO: 270
  158cShortMainM20

SEQ ID NO: 365 - DNA, 40 bp, Artificial Sequence; identical to SEQ ID NO: 271
  161cLong

SEQ ID NO: 366 - DNA, 73 bp, Artificial Sequence; identical to SEQ ID NO: 272
  162sBothLongM20

SEQ ID NO: 367 - DNA, 16 bp, Artificial Sequence
  SmBiT-95w
aaggaattgaggaagg

SEQ ID NO: 368 - DNA, 16 bp, Artificial Sequence
  LgBiT-138w
atccgcgacctgctcc